European Patent Application EP 4 700 132 A1, published February 25, 2026. Title: DETECTION METHOD FOR TARGET ecDNA AND DETECTION KIT FOR TARGET ecDNA. Applicant: CANON MEDICAL SYSTEMS CORPORATION. Application EP. The sequence listing filed with the application follows.

SEQUENCE LISTING (10 sequences)

SEQ ID NO: 1 - DNA, 20 bp, synthetic construct
  source 1..20: mol_type = other DNA
cttcggggagacaacgacgg

SEQ ID NO: 2 - DNA, 20 bp, synthetic construct
  source 1..20: mol_type = other DNA
ccggttttcggggctttatc

SEQ ID NO: 3 - DNA, 20 bp, synthetic construct
  source 1..20: mol_type = other DNA
ccctattcgctccggatctc

SEQ ID NO: 4 - DNA, 20 bp, synthetic construct
  source 1..20: mol_type = other DNA
caagaggcgaacacacaacg

SEQ ID NO: 5 - DNA, 20 bp, synthetic construct
  source 1..20: mol_type = other DNA
caactccgggatctggtcac

SEQ ID NO: 6 - DNA, 19 bp, synthetic construct
  source 1..19: mol_type = other DNA
ctcctacgttgcggtcaca

SEQ ID NO: 7 - DNA, 19 bp, synthetic construct
  source 1..19: mol_type = other DNA
tccgggtcgcagatgaaac

SEQ ID NO: 8 - DNA, 29 bp, synthetic construct
  source 1..29: mol_type = other DNA
tgtagtaattccagcgagaggcagaggga

SEQ ID NO: 9 - DNA, 28 bp, synthetic construct
  source 1..28: mol_type = other DNA
gttttagctcgttcctcctctggcgctc

SEQ ID NO: 10 - DNA, 27 bp, synthetic construct
  source 1..27: mol_type = other DNA
gttcaccatgtctcctcccagcagctc